European Patent Specification EP 3 807 297 B1, published October 22, 2025. Title: SYNTHETIC LIVER-TROPIC ADENO-ASSOCIATED VIRUS CAPSIDS AND USES THEREOF. Applicant: The University of North Carolina at Chapel Hill Xiao, Xiao Li, Juan Xiao, Bin Yuan, Zhenhua. The sequence listing filed with the application follows.

SEQUENCE LISTING (8 sequences)

SEQ ID NO: 1 - DNA, 2214 bp, Artificial
  AAVXL12 capsid gene DNA sequence
atggctgccgatggttatcttccagattggctcgaggacaacctctctgagggcattcgcgagtggtgggcgctgaaacctggagccccgaagcccaaagccaaccagcaaaagcaggacgacggccggggtctggtgcttcctggctacaagtacctcggacccttcaacggactcgacaagggggagcccgtcaacgcggcggacgcagcggccctggagcacgacaaggcctacgaccagcagctgcaggcgggtgacaatccgtacctgcggtataaccacgccgacgccgagtttcaggagcgtctgcaagaagatacgtcttttgggggcaacctcgggcgagcagtcttccaggccaagaagcgggttctcgaacctctcggtctggttgaggaaggcgctaagacggctcctggaaagaagagaccggtagagccatcaccccagcgttctccagactcctctacgggcatcggcaagaaaggccaacagcccgccagaaaaagactcaattttggtcagactggcgactcagagtcagttccagaccctcaacctctcggagaacctccagcagcgccctctggtgtgggacctaatacaatggcttcaggcggtggcgcaccaatggcagacaataacgaaggcgcctccggagtgggtaatgcctcaggaaattggcattgcgattccacatggctgggcgacagagtcatcaccaccagcacccgaacatgggccttgcccacctacaacaatcacctctacaagcaaatctccagtgcttcaacgggggccagcaacgacaaccactacttcggctacagcaccccctgggggtattttgatttcaacagattccactgccacttttcaccacgtgactggcagcgactcatcaacaacaattggggattccggcccaagagactcaacttcaaactcttcaacatccaagtcaaggaggtcacgacgaatgatggcgtcacgaccatcgctaataaccttaccagcacggttcaagtcttctcggactcggagtaccagttgccgtacgtcctcggctctgcgcaccagggctgcctccctccgttcccggcggacgtgttcatgattccgcagtacggctacctaacgctcaacaatggcagccaggcagtgggacggtcatccttttactgcctggaatatttcccatcgcagatgctgagaacgggcaacaactttaccttcagctacacctttgaggaagtgcctttccacagcagctacgcgcacagccagagcctggaccggctgatgaatcctctcatcgaccaatacctgtattacctgaacagaactcaaaatcagtccggaagtgcccaaaacaaggacttgctgtttagccgtgggtctccagctggcatgtctgttcagcccaaaaactggctacctggaccctgttaccggcagcagcgcgtttctaaaacaaaaacagacaacaacaacagcaactttacctggactggtgcttcaaaatataaccttaatgggcgtgaatctataatcaaccctggcactgctatggcctcacacaaagacgacaaagacaagttctttcccatgagcggtgtcatgatttttggaaaggagagcgccggagcttcaaacactgcattggacaatgtcatgatcacagacgaagaggaaatcaaagccactaaccccgtggccaccgaaagatttgggactgtggcagtcaatctccagagcagcagcacagaccctgcgaccggagatgtgcatgttatgggagccttacctggaatggtgtggcaagacagagacgtatacctgcagggtcctatttgggccaaaattcctcacacggatggacactttcacccgtctcctcttatgggcggctttggactcaagaacccgcctcctcagatcctcatcaaaaacacgcctgttcctgcgaatcctccggcagagttttcggctacaaagtttgcttcattcatcacccagtattccacaggacaagtgagcgtggagattgaatgggagctgcagaaagaaaacagcaaacgctggaatcccgaagtgcagtatacatctaactatgcaaaatctgccaacgttgatttcactgtggacaacaatggactttatactgagcctcgccccattggcacccgttacctcacccgtcccctgtaa

SEQ ID NO: 2 - DNA, 2214 bp, Artificial
  AAVXL32 capsid gene DNA sequence
atggctgccgatggttatcttccagattggctcgaggacaacctctctgagggcattcgcgagtggtgggcgctgaaacctggagccccgaagcccaaagccaaccagcaaaagcaggacgacggccggggtctggtgcttcctggctacaagtacctcggacccttcaacggactcgacaagggggagcccgtcaacgcggcggacgcagcggccctggagcacgacaaggcctacgaccagcagctgcaggcgggtgacaatccgtacctgcggtataaccacgccgacgccgagtttcaggagcgtctgcaagaagatacgtcttttgggggcaacctcgggcgagcagtcttccaggccaagaagcgggttctcgaacctctcggtctggttgaggaaggcgctaagacggctcctggaaagaagagaccggtagagccatcaccccagcgttctccagactcctctacgggcatcggcaagaaaggccaacagcccgccagaaaaagactcaattttggtcagactggcgactcagagtcagttccagaccctcaacctctcggagaacctccagcagcgccctctggtgtgggacctaatacaatggcttcaggcggtggcgcaccaatggcagacaataacgaaggcgccgacggagtgggtaatgcctcaggaaattggcattgcgattccacatggctgggcgacagagtcatcaccaccagcacccgaacatgggccttgcccacctataacaaccacctctacaagcaaatctccagtgcttcaacgggggccagcaacgacaaccactacttcggctacagcaccccctgggggtattttgatttcaacagattccactgccatttctcaccacgtgactggcagcgactcatcaacaacaattggggattccggcccaagagactcaacttcaagctcttcaacatccaagtcaaggaggtcacgacgaatgatggcgtcacgaccatcgctaataaccttaccagcacggttcaagtcttctcggactcggagtaccagttgccgtacgtcctcggctctgcgcaccagggctgcctccctccgttcccggcggacgtgttcatgattccgcaatacggctacctgacgctcaacaatggcagccaagccgtgggacgttcatccttttactgcctggaatatttcccttctcagatgctgagaacgggcaacaactttaccttcagctacacctttgaggaagtgcctttccacagcagctacgcgcacagccagagcctggaccggctgatgaatcctctcatcgaccagtacctgtattacctgaacagaactcagaatcagtccggaagtgcccaaaacaaggacttgctgtttagccgtgggtctccagctggcatgtctgttcagcccaaaaactggctacctggaccctgttaccggcagcagcgcgtttctaaaacaaaaacagacaacaacaacagcaactttacctggactggtgcttcaaaatataacctcaatgggcgtgaatccatcatcaaccctggcactgctatggcctcacacaaagacgacaaagacaagttctttcccatgagcggtgtcatgatttttggaaaggagagcgccggagcttcaaacactgcattggacaatgtcatgatcacagacgaagaggaaatcaaagccactaaccccgtggccaccgaaagatttgggactgtggcagtcaatctccagagcagcagcacagaccctgcgaccggagatgtgcatgttatgggagccttacctggaatggtgtggcaagacagagacgtatacctgcagggtcctatttgggccaaaattcctcacacggatggacactttcacccgtctcctctcatgggcggctttggacttaagcacccgcctcctcagatcctcatcaaaaacacgcctgttcctgcgaatcctccggcagagttttcggctacaaagtttgcttcattcatcacccagtattccacaggacaagtgagcgtggagattgaatgggagctgcagaaagaaaacagcaaacgctggaatcccgaagtgcagtatacatctaactatgcaaaatctgccaacgttgattttactgtggacaacaatggactttatactgagcctcgccccattggcacccgttacctcacccgtcccctgtaa

SEQ ID NO: 3 - DNA, 2214 bp, Artificial
  AAVXL32.1 capsid gene DNA sequence
atggctgccgatggttatcttccagattggctcgaggacaacctctctgagggcattcgcgagtggtgggcgctgaaacctggagccccgaagcccaaagccaaccagcaaaagcaggacgacggccggggtctggtgcttcctggctacaagtacctcggacccttcaacggactcgacaagggggagcccgtcaacgcggcggacgcagcggccctcgagcacgacaaggcctacgaccagcagctgcaggcgggtgacaatccgtacctgcggtataaccacgccgacgccgagtttcaggagcgtctgcaagaagatacgtcttttgggggcaacctcgggcgagcagtcttccaggccaagaagcgggttctcgaacctctcggtctggttgaggaaggcgctaagacggctcctggaaagaagagaccggtagagccatcaccccagcgttctccagactcctctacgggcatcggcaagaaaggccaacagcccgccagaaaaagactcaattttggtcagactggcgactcagagtcagttccagaccctcaacctctcggagaacctccagcagcgccctctggtgtgggacctaatacaatggcttcaggcggtggcgcaccaatggcagacaataacgaaggcgccgacggagtgggtaatgcctcaggaaattggcattgcgattccacatggctgggcgacagagtcatcaccaccagcacccgaacatgggccttgcccacctataacaaccacctctacaagcaaatctccagtgcttcaacgggggccagcaacgacaaccactacttcggctacagcaccccctgggggtattttgatttcaacagattccactgccatttctcaccacgtgactggcagcgactcatcaacaacaattggggattccggcccaagagactcaacttcaagctcttcaacatccaagtcaaggaggtcacgacgaatgatggcgtcacgaccatcgctaataaccttaccagcacggttcaagtcttctcggactcggagtaccagttgccgtacgtcctcggctctgcgcaccagggctgcctccctccgttcccggcggacgtgttcatgattccgcaatacggctacctgacgctcaacaatggcagccaagccgtgggacgttcatccttttactgcctggaatatttcccttctcagatgctgagaacgggcaacaactttaccttcagctacacctttgaggaagtgcctttccacagcagctacgcgcacagccagagcctggaccggctgatgaatcctctcatcgaccagtacctgtattacctgaacagaactcagaatcagtccggaagtgcccaaaacaaggacttgctgtttagccgtgggtctccagctggcatgtctgttcagcccaaaaactggctacctggaccctgttaccggcagcagcgcgtttctaaaacaaaaacagacaacaacaacagcaactttacctggactggtgcttcaaaatataacctcaatgggcgtgaatccatcatcaaccctggcactgctatggcctcacacaaagacgacaaagacaagttctttcccatgagcggtgtcatgatttttggaaaggagagcgccggagcttcaaacactgcattggacaatgtcatgatcacagacgaagaggaaatcaaagccactaaccccgtggccaccgaaagatttgggactgtggcagtcaatctccagagcagcagcacagaccctgcgaccggagatgtgcatgttatgggagccttacctggaatggtgtggcaagacagagacgtatacctgcagggtcctatttgggccaaaattcctcacacggatggacactttcacccgtctcctctcatgggcggctttggacttaagcacccgcctcctcagatcctcatcaaaaacacgcctgttcctgcgaatcctccggcagagttttcggctacaaagtttgcttcattcatcacccagtattccacaggacaagtgagcgtggagattgaatgggagctgcagaaagaaaacagcaaacgctggaatcccgaagtgcagtatacatctaactatgcaaaatctgccaacgttgattttactgtggacaacaatggactttatactgagcctcgccccattggcacccgttacctcacccgtcccctgtaa

SEQ ID NO: 4 - protein, 737 aa, Artificial
  AAVXL12 capsid amino acid sequence
MAADGYLPDWLEDNLSEGIREWWALKPGAPKPKANQQKQDDGRGLVLPGYKYLGPFNGLDKGEPVNAADAAALEHDKAYDQQLQAGDNPYLRYNHADAEFQERLQEDTSFGGNLGRAVFQAKKRVLEPLGLVEEGAKTAPGKKRPVEPSPQRSPDSSTGIGKKGQQPARKRLNFGQTGDSESVPDPQPLGEPPAAPSGVGPNTMASGGGAPMADNNEGASGVGNASGNWHCDSTWLGDRVITTSTRTWALPTYNNHLYKQISSASTGASNDNHYFGYSTPWGYFDFNRFHCHFSPRDWQRLINNNWGFRPKRLNFKLFNIQVKEVTTNDGVTTIANNLTSTVQVFSDSEYQLPYVLGSAHQGCLPPFPADVFMIPQYGYLTLNNGSQAVGRSSFYCLEYFPSQMLRTGNNFTFSYTFEEVPFHSSYAHSQSLDRLMNPLIDQYLYYLNRTQNQSGSAQNKDLLFSRGSPAGMSVQPKNWLPGPCYRQQRVSKTKTDNNNSNFTWTGASKYNLNGRESIINPGTAMASHKDDKDKFFPMSGVMIFGKESAGASNTALDNVMITDEEEIKATNPVATERFGTVAVNLQSSSTDPATGDVHVMGALPGMVWQDRDVYLQGPIWAKIPHTDGHFHPSPLMGGFGLKNPPPQILIKNTPVPANPPAEFSATKFASFITQYSTGQVSVEIEWELQKENSKRWNPEVQYTSNYAKSANVDFTVDNNGLYTEPRPIGTRYLTRPL

SEQ ID NO: 5 - protein, 737 aa, Artificial
  AAVXL32 capsid amino acid sequence
MAADGYLPDWLEDNLSEGIREWWALKPGAPKPKANQQKQDDGRGLVLPGYKYLGPFNGLDKGEPVNAADAAALEHDKAYDQQLQAGDNPYLRYNHADAEFQERLQEDTSFGGNLGRAVFQAKKRVLEPLGLVEEGAKTAPGKKRPVEPSPQRSPDSSTGIGKKGQQPARKRLNFGQTGDSESVPDPQPLGEPPAAPSGVGPNTMASGGGAPMADNNEGADGVGNASGNWHCDSTWLGDRVITTSTRTWALPTYNNHLYKQISSASTGASNDNHYFGYSTPWGYFDFNRFHCHFSPRDWQRLINNNWGFRPKRLNFKLFNIQVKEVTTNDGVTTIANNLTSTVQVFSDSEYQLPYVLGSAHQGCLPPFPADVFMIPQYGYLTLNNGSQAVGRSSFYCLEYFPSQMLRTGNNFTFSYTFEEVPFHSSYAHSQSLDRLMNPLIDQYLYYLNRTQNQSGSAQNKDLLFSRGSPAGMSVQPKNWLPGPCYRQQRVSKTKTDNNNSNFTWTGASKYNLNGRESIINPGTAMASHKDDKDKFFPMSGVMIFGKESAGASNTALDNVMITDEEEIKATNPVATERFGTVAVNLQSSSTDPATGDVHVMGALPGMVWQDRDVYLQGPIWAKIPHTDGHFHPSPLMGGFGLKHPPPQILIKNTPVPANPPAEFSATKFASFITQYSTGQVSVEIEWELQKENSKRWNPEVQYTSNYAKSANVDFTVDNNGLYTEPRPIGTRYLTRPL

SEQ ID NO: 6 - protein, 737 aa, Artificial; identical to SEQ ID NO: 5
  AAV XL32.1 capsid amino acid sequence

SEQ ID NO: 7 - DNA, 35 bp, Artificial
  DNA Primer CAP-5'
cccaagcttcgatcaactacgcagacaggtaccaa

SEQ ID NO: 8 - DNA, 41 bp, Artificial
  DNA Primer CAP-3'
ataagaatgcggccgcagagaccaaagttcaactgaaacga